European Patent Specification EP 3 334 745 B1, published May 15, 2024. Title: CYCLIC DI-NUCLEOTIDE COMPOUNDS AS STING AGONISTS. Applicant: MERCK SHARP & DOHME CORP. The sequence listing filed with the application follows.

SEQUENCE LISTING (5 sequences)

SEQ ID NO: 1 - protein, 475 aa, Unknown
  cGAS enzyme
MAHHHHHHGSDSEVNQEAKPEVKPEVKPETHINLKVSDGSSEIFFKIKKTTPLRRLMEAFAKRQGKEMDSLTFLYDGIEIQADQTPEDLDMEDNDIIEAHREQIGGENLYFQGGASKLRAVLEKLKLSRDDISTAAGMVKGVVDHLLLRLKCDSAFRGVGLLNTGSYYEHVKISAPNEFDVMFKLEVPRIQLEEYSNTRAYYFVKFKRNPKENPLSQFLEGEILSASKMLSKFRKIIKEEINDIKDTDVIMKRKRGGSPAVTLLISEKISVDITLALESKSSWPASTQEGLRIQNWLSAKVRKQLRLKPFYLVPKHAKEGNGFQEETWRLSFSHIEKEILNNHGKSKTCCENKEEKCCRKDCLKLMKYLLEQLKERFKDKKHLDKFSSYHVKTAFFHVCTQNPQDSQWDRKDLGLCFDNCVTYFLQCLRTEKLENYFIPEFNLFSSNLIDKRSKEFLTKQIEYERNNEFPVFDEF

SEQ ID NO: 2 - protein, 414 aa, Homo Sapien
MPHSSLHPSIPCPRGHGAQKAALVLLSACLVTLWGLGEPPEHTLRYLVLHLASLQLGLLLNGVCSLAEELHHIHSRYRGSYWRTVRACLGCPLRRGALLLLSIYFYYSLPNAVGPPFTWMLALLGLSQALNILLGLKGLAPAEISAVCEKGNFNVAHGLAWSYYIGYLRLILPELQARIRTYNQHYNNLLRGAVSQRLYILLPLDCGVPDNLSMADPNIRFLDKLPQQTADRAGIKDRVYSNSIYELLENGQRAGTCVLEYATPLQTLFAMSQYSQAGFSREDRLEQAKLFCQTLEDILADAPESQNNCRLIAYQEPADDSSFSLSQEVLRHLRQEEKEEVTVGSLKTSAVPSTSTMSQEPELLISGMEKPLPLRTDFSGGGLNDIFEAQKIEWHEGSLEVLFQGPHHHHHHHH

SEQ ID NO: 3 - DNA, 6482 bp, Homo Sapien
ggaacggctccgcccactattaatgaaattaaaaattccaattttaaaaaacgcagcaagagaaacatttgtatgaaagaatgcgtagaaggaaagaaaaatgtcgtcgacatgctgaacaacaagattaatatgcctccgtgtataaaaaaaatattgaacgatttgaaagaaaacaatgtaccgcgcggcggtatgtacaggaagaggtttatactaaactgttacattgcaaacgtggtttcgtgtgccaagtgtgaaaaccgatgtttaatcaaggctctgacgcatttctacaaccacgactccaagtgtgtgggtgaagtcatgcatcttttaatcaaatcccaagatgtgtataaaccaccaaactgccaaaaaatgaaaactgtcgacaagctctgtccgtttgctggcaactgcaagggtctcaatcctatttgtaattattgaataataaaacaattataaatgctaaatttgttttttattaacgatacaaaccaaacgcaacaagaacatttgtagtattatctataattgaaaacgcgtagttataatcgctgaggtaatatttaaaatcattttcaaatgattcacagttaatttgcgacaatataattttattttcacataaactagacgccttgtcgtcttcttcttcgtattccttctctttttcatttttctcttcataaaaattaacatagttattatcgtatccatatatgtatctatcgtatagagtaaattttttgttgtcataaatatatatgtcttttttaatggggtgtatagtaccgctgcgcatagtttttctgtaatttacaacagtgctattttctggtagttcttcggagtgtgttgctttaattattaaatttatataatcaatgaatttgggatcgtcggttttgtacaatatgttgccggcatagtacgcagcttcttctagttcaattacaccattttttagcagcaccggattaacataactttccaaaatgttgtacgaaccgttaaacaaaaacagttcacctcccttttctatactattgtctgcgagcagttgtttgttgttaaaaataacagccattgtaatgagacgcacaaactaatatcacaaactggaaatgtctatcaatatatagttgctgatcagatctgatcatggagataattaaaatgataaccatctcgcaaataaataagtattttactgttttcgtaacagttttgtaataaaaaaacctataaatataggatccatgccccactccagcctgcatccatccatcccgtgtcccaggggtcacggggcccagaaggcagccttggttctgctgagtgcctgcctggtgaccctttgggggctaggagagccaccagagcacactctccggtacctggtgctccacctagcctccctgcagctgggactgctgttaaacggggtctgcagcctggctgaggagctgcaccacatccactccaggtaccggggcagctactggaggactgtgcgggcctgcctgggctgccccctccgccgtggggccctgttgctgctgtccatctatttctactactccctcccaaatgcggtcggcccgcccttcacttggatgcttgccctcctgggcctctcgcaggcactgaacatcctcctgggcctcaagggcctggccccagctgagatctctgcagtgtgtgaaaaagggaatttcaacgtggcccatgggctggcatggtcatattacatcggatatctgcggctgatcctgccagagctccaggcccggattcgaacttacaatcagcattacaacaacctgctacggggtgcagtgagccagcggctgtatattctcctcccattggactgtggggtgcctgataacctgagtatggctgaccccaacattcgcttcctggataaactgccccagcagaccgctgaccgtgctggcatcaaggatcgggtttacagcaacagcatctatgagcttctggagaacgggcagcgggcgggcacctgtgtcctggagtacgccacccccttgcagactttgtttgccatgtcacaatacagtcaagctggctttagccgggaggataggcttgagcaggccaaactcttctgccagacacttgaggacatcctggcagatgcccctgagtctcagaacaactgccgcctcattgcctaccaggaacctgcagatgacagcagcttctcgctgtcccaggaggttctccggcacctgcggcaggaggaaaaggaagaggttactgtgggcagcttgaagacctcagcggtgcccagtacctccacgatgtcccaagagcctgagctcctcatcagtggaatggaaaagcccctccctctccgcacggatttctctggcggtggcctgaacgacatcttcgaagcccagaaaatcgaatggcatgaaggcagcctggaagtgctgttccagggcccacaccaccatcatcaccatcaccattaatgagcggccgcactcgagcaccaccaccaccaccactaacctaggtagctgagcgcatgcaagctgatccgggttattagtacatttattaagcgctagattctgtgcgttgttgatttacagacaattgttgtacgtattttaataattcattaaatttataatctttagggtggtatgttagagcgaaaatcaaatgattttcagcgtctttatatctgaatttaaatattaaatcctcaatagatttgtaaaataggtttcgattagtttcaaacaagggttgtttttccgaaccgatggctggactatctaatggattttcgctcaacgccacaaaacttgccaaatcttgtagcagcaatctagctttgtcgatattcgtttgtgttttgttttgtaataaaggttcgacgtcgttcaaaatattatgcgcttttgtatttctttcatcactgtcgttagtgtacaattgactcgacgtaaacacgttaaatagagcttggacatatttaacatcgggcgtgttagctttattaggccgattatcgtcgtcgtcccaaccctcgtcgttagaagttgcttccgaagacgattttgccatagccacacgacgcctattaattgtgtcggctaacacgtccgcgatcaaatttgtagttgagctttttggaattatttctgattgcgggcgtttttgggcgggtttcaatctaactgtgcccgattttaattcagacaacacgttagaaagcgatggtgcaggcggtggtaacatttcagacggcaaatctactaatggcggcggtggtggagctgatgataaatctaccatcggtggaggcgcaggcggggctggcggcggaggcggaggcggaggtggtggcggtgatgcagacggcggtttaggctcaaatgtctctttaggcaacacagtcggcacctcaactattgtactggtttcgggcgccgtttttggtttgaccggtctgagacgagtgcgatttttttcgtttctaatagcttccaacaattgttgtctgtcgtctaaaggtgcagcgggttgaggttccgtcggcattggtggagcgggcggcaattcagacatcgatggtggtggtggtggtggaggcgctggaatgttaggcacgggagaaggtggtggcggcggtgccgccggtataatttgttctggtttagtttgttcgcgcacgattgtgggcaccggcgcaggcgccgctggctgcacaacggaaggtcgtctgcttcgaggcagcgcttggggtggtggcaattcaatattataattggaatacaaatcgtaaaaatctgctataagcattgtaatttcgctatcgtttaccgtgccgatatttaacaaccgctcaatgtaagcaattgtattgtaaagagattgtctcaagctcggatcgatcccgcacgccgataacaagccttttcatttttactacagcattgtagtggcgagacacttcgctgtcgtcgaggtttaaacgcttcctcgctcactgactcgctgcgctcggtcgttcggctgcggcgagcggtatcagctcactcaaaggcggtaatacggttatccacagaatcaggggataacgcaggaaagaacatgtgagcaaaaggccagcaaaaggccaggaaccgtaaaaaggccgcgttgctggcgtttttccataggctccgcccccctgacgagcatcacaaaaatcgacgctcaagtcagaggtggcgaaacccgacaggactataaagataccaggcgtttccccctggaagctccctcgtgcgctctcctgttccgaccctgccgcttaccggatacctgtccgcctttctcccttcgggaagcgtggcgctttctcatagctcacgctgtaggtatctcagttcggtgtaggtcgttcgctccaagctgggctgtgtgcacgaaccccccgttcagcccgaccgctgcgccttatccggtaactatcgtcttgagtccaacccggtaagacacgacttatcgccactggcagcagccactggtaacaggattagcagagcgaggtatgtaggcggtgctacagagttcttgaagtggtggcctaactacggctacactagaaggacagtatttggtatctgcgctctgctgaagccagttaccttcggaaaaagagttggtagctcttgatccggcaaacaaaccaccgctggtagcggtggtttttttgtttgcaagcagcagattacgcgcagaaaaaaaggatctcaagaagatcctttgatcttttctacggggtctgacgctcagtggaacgaaaactcacgttaagggattttggtcatgagattatcaaaaaggatcttcacctagatccttttaaattaaaaatgaagttttaaatcaatctaaagtatatatgagtaaacttggtctgacagttaccaatgcttaatcagtgaggcacctatctcagcgatctgtctatttcgttcatccatagttgcctgactccccgtcgtgtagataactacgatacgggagggcttaccatctggccccagtgctgcaatgataccgcgagacccacgctcaccggctccagatttatcagcaataaaccagccagccggaagggccgagcgcagaagtggtcctgcaactttatccgcctccatccagtctattaattgttgccgggaagctagagtaagtagttcgccagttaatagtttgcgcaacgttgttgccattgctacaggcatcgtggtgtcacgctcgtcgtttggtatggcttcattcagctccggttcccaacgatcaaggcgagttacatgatcccccatgttgtgcaaaaaagcggttagctccttcggtcctccgatcgttgtcagaagtaagttggccgcagtgttatcactcatggttatggcagcactgcataattctcttactgtcatgccatccgtaagatgcttttctgtgactggtgagtactcaaccaagtcattctgagaatagtgtatgcggcgaccgagttgctcttgcccggcgtcaatacgggataataccgcgccacatagcagaactttaaaagtgctcatcattggaaaacgttcttcggggcgaaaactctcaaggatcttaccgctgttgagatccagttcgatgtaacccactcgtgcacccaactgatcttcagcatcttttactttcaccagcgtttctgggtgagcaaaaacaggaaggcaaaatgccgcaaaaaagggaataagggcgacacggaaatgttgaatactcatactcttcctttttcaatattattgaagcatttatcagggttattgtctcatgagcggatacatatttgaatgtatttagaaaaataaacaaataggggttccgcgcacatttccccgaaaagtgccacctgacgcgccctgtagcggcgcattaagcgcggcgggtgtggtggttacgcgcagcgtgaccgctacacttgccagcgccctagcgcccgctcctttcgctttcttcccttcctttctcgccacgttcgccggctttccccgtcaagctctaaatcgggggctccctttagggttccgatttagtgctttacggcacctcgaccccaaaaaacttgattagggtgatggttcacgtagtgggccatcgccctgatagacggtttttcgccctttgacgttggagtccacgttctttaatagtggactcttgttccaaactggaacaacactcaaccctatctcggtctattcttttgatttataagggattttgccgatttcggcctattggttaaaaaatgagctgatttaacaaaaatttaacgcgaattttaacaaaatattaacgtttacaatttcccattcgccattcaggctgcgcaactgttgggaagggcgatcggtgcgggcctcttcgctattacgcca

SEQ ID NO: 4 - protein, 414 aa, Homo Sapien
MPHSSLHPSIPCPRGHGAQKAALVLLSACLVTLWGLGEPPEHTLRYLVLHLASLQLGLLLNGVCSLAEELRHIHSRYRGSYWRTVRACLGCPLRRGALLLLSIYFYYSLPNAVGPPFTWMLALLGLSQALNILLGLKGLAPAEISAVCEKGNFNVAHGLAWSYYIGYLRLILPELQARIRTYNQHYNNLLRGAVSQRLYILLPLDCGVPDNLSMADPNIRFLDKLPQQTGDRAGIKDRVYSNSIYELLENGQRAGTCVLEYATPLQTLFAMSQYSQAGFSREDRLEQAKLFCRTLEDILADAPESQNNCRLIAYQEPADDSSFSLSQEVLRHLRQEEKEEVTVGSLKTSAVPSTSTMSQEPELLISGMEKPLPLRTDFSGGGLNDIFEAQKIEWHEGSLEVLFQGPHHHHHHHH

SEQ ID NO: 5 - DNA, 6482 bp, Homo Sapien
ggaacggctccgcccactattaatgaaattaaaaattccaattttaaaaaacgcagcaagagaaacatttgtatgaaagaatgcgtagaaggaaagaaaaatgtcgtcgacatgctgaacaacaagattaatatgcctccgtgtataaaaaaaatattgaacgatttgaaagaaaacaatgtaccgcgcggcggtatgtacaggaagaggtttatactaaactgttacattgcaaacgtggtttcgtgtgccaagtgtgaaaaccgatgtttaatcaaggctctgacgcatttctacaaccacgactccaagtgtgtgggtgaagtcatgcatcttttaatcaaatcccaagatgtgtataaaccaccaaactgccaaaaaatgaaaactgtcgacaagctctgtccgtttgctggcaactgcaagggtctcaatcctatttgtaattattgaataataaaacaattataaatgtcaaatttgttttttattaacgatacaaaccaaacgcaacaagaacatttgtagtattatctataattgaaaacgcgtagttataatcgctgaggtaatatttaaaatcattttcaaatgattcacagttaatttgcgacaatataattttattttcacataaactagacgccttgtcgtcttcttcttcgtattccttctctttttcatttttctcttcataaaaattaacatagttattatcgtatccatatatgtatctatcgtatagagtaaattttttgttgtcataaatatatatgtcttttttaatggggtgtatagtaccgctgcgcatagtttttctgtaatttacaacagtgctattttctggtagttcttcggagtgtgttgctttaattattaaatttatataatcaatgaatttgggatcgtcggttttgtacaatatgttgccggcatagtacgcagcttcttctagttcaattacaccattttttagcagcaccggattaacataactttccaaaatgttgtacgaaccgttaaacaaaaacagttcacctcccttttctatactattgtctgcgagcagttgtttgttgttaaaaataacagccattgtaatgagacgcacaaactaatatcacaaactggaaatgtctatcaatatatagttgctgatcagatctgatcatggagataattaaaatgataaccatctcgcaaataaataagtattttactgttttcgtaacagttttgtaataaaaaaacctataaatataggatccatgccccactccagcctgcatccatccatcccgtgtcccaggggtcacggggcccagaaggcagccttggttctgctgagtgcctgcctggtgaccctttgggggctaggagagccaccagagcacactctccggtacctggtgctccacctagcctccctgcagctgggactgctgttaaacggggtctgcagcctggctgaggagctgcgccacatccactccaggtaccggggcagctactggaggactgtgcgggcctgcctgggctgccccctccgccgtggggccctgttgctgctgtccatctatttctactactccctcccaaatgcggtcggcccgcccttcacttggatgcttgccctcctgggcctctcgcaggcactgaacatcctcctgggcctcaagggcctggccccagctgagatctctgcagtgtgtgaaaaagggaatttcaacgtggcccatgggctggcatggtcatattacatcggatatctgcggctgatcctgccagagctccaggcccggattcgaacttacaatcagcattacaacaacctgctacggggtgcagtgagccagcggctgtatattctcctcccattggactgtggggtgcctgataacctgagtatggctgaccccaacattcgcttcctggataaactgccccagcagaccggtgaccgtgctggcatcaaggatcgggtttacagcaacagcatctatgagcttctggagaacgggcagcgggcgggcacctgtgtcctggagtacgccacccccttgcagactttgtttgccatgtcacaatacagtcaagctggctttagccgggaggataggcttgagcaggccaaactcttctgccggacacttgaggacatcctggcagatgcccctgagtctcagaacaactgccgcctcattgcctaccaggaacctgcagatgacagcagcttctcgctgtcccaggaggttctccggcacctgcggcaggaggaaaaggaagaggttactgtgggcagcttgaagacctcagcggtgcccagtacctccacgatgtcccaagagcctgagctcctcatcagtggaatggaaaagcccctccctctccgcacggatttctctggcggtggcctgaacgacatcttcgaagcccagaaaatcgaatggcatgaaggcagcctggaagtgctgttccagggcccacaccaccatcatcaccatcaccattaatgagcggccgcactcgagcaccaccaccaccaccactaacctaggtagctgagcgcatgcaagctgatccgggttattagtacatttattaagcgctagattctgtgcgttgttgatttacagacaattgttgtacgtattttaataattcattaaatttataatctttagggtggtatgttagagcgaaaatcaaatgattttcagcgtctttatatctgaatttaaatattaaatcctcaatagatttgtaaaataggtttcgattagtttcaaacaagggttgtttttccgaaccgatggctggactatctaatggattttcgctcaacgccacaaaacttgccaaatcttgtagcagcaatctagctttgtcgatattcgtttgtgttttgttttgtaataaaggttcgacgtcgttcaaaatattatgcgcttttgtatttctttcatcactgtcgttagtgtacaattgactcgacgtaaacacgttaaatagagcttggacatatttaacatcgggcgtgttagctttattaggccgattatcgtcgtcgtcccaaccctcgtcgttagaagttgcttccgaagacgattttgccatagccacacgacgcctattaattgtgtcggctaacacgtccgcgatcaaatttgtagttgagctttttggaattatttctgattgcgggcgtttttgggcgggtttcaatctaactgtgcccgattttaattcagacaacacgttagaaagcgatggtgcaggcggtggtaacatttcagacggcaaatctactaatggcggcggtggtggagctgatgataaatctaccatcggtggaggcgcaggcggggctggcggcggaggcggaggcggaggtggtggcggtgatgcagacggcggtttaggctcaaatgtctctttaggcaacacagtcggcacctcaactattgtactggtttcgggcgccgtttttggtttgaccggtctgagacgagtgcgatttttttcgtttctaatagcttccaacaattgttgtctgtcgtctaaaggtgcagcgggttgaggttccgtcggcattggtggagcgggcggcaattcagacatcgatggtggtggtggtggtggaggcgctggaatgttaggcacgggagaaggtggtggcggcggtgccgccggtataatttgttctggtttagtttgttcgcgcacgattgtgggcaccggcgcaggcgccgctggctgcacaacggaaggtcgtctgcttcgaggcagcgcttggggtggtggcaattcaatattataattggaatacaaatcgtaaaaatctgctataagcattgtaatttcgctatcgtttaccgtgccgatatttaacaaccgctcaatgtaagcaattgtattgtaaagagattgtctcaagctcggatcgatcccgcacgccgataacaagccttttcatttttactacagcattgtagtggcgagacacttcgctgtcgtcgaggtttaaacgcttcctcgctcactgactcgctgcgctcggtcgttcggctgcggcgagcggtatcagctcactcaaaggcggtaatacggttatccacagaatcaggggataacgcaggaaagaacatgtgagcaaaaggccagcaaaaggccaggaaccgtaaaaaggccgcgttgctggcgtttttccataggctccgcccccctgacgagcatcacaaaaatcgacgctcaagtcagaggtggcgaaacccgacaggactataaagataccaggcgtttccccctggaagctccctcgtgcgctctcctgttccgaccctgccgcttaccggatacctgtccgcctttctcccttcgggaagcgtggcgctttctcatagctcacgctgtaggtatctcagttcggtgtaggtcgttcgctccaagctgggctgtgtgcacgaaccccccgttcagcccgaccgctgcgccttatccggtaactatcgtcttgagtccaacccggtaagacacgacttatcgccactggcagcagccactggtaacaggattagcagagcgaggtatgtaggcggtgctacagagttcttgaagtggtggcctaactacggctacactagaaggacagtatttggtatctgcgctctgctgaagccagttaccttcggaaaaagagttggtagctcttgatccggcaaacaaaccaccgctggtagcggtggtttttttgtttgcaagcagcagattacgcgcagaaaaaaaggatctcaagaagatcctttgatcttttctacggggtctgacgctcagtggaacgaaaactcacgttaagggattttggtcatgagattatcaaaaaggatcttcacctagatccttttaaattaaaaatgaagttttaaatcaatctaaagtatatatgagtaaacttggtctgacagttaccaatgcttaatcagtgaggcacctatctcagcgatctgtctatttcgttcatccatagttgcctgactccccgtcgtgtagataactacgatacgggagggcttaccatctggccccagtgctgcaatgataccgcgagacccacgctcaccggctccagatttatcagcaataaaccagccagccggaagggccgagcgcagaagtggtcctgcaactttatccgcctccatccagtctattaattgttgccgggaagctagagtaagtagttcgccagttaatagtttgcgcaacgttgttgccattgctacaggcatcgtggtgtcacgctcgtcgtttggtatggcttcattcagctccggttcccaacgatcaaggcgagttacatgatcccccatgttgtgcaaaaaagcggttagctccttcggtcctccgatcgttgtcagaagtaagttggccgcagtgttatcactcatggttatggcagcactgcataattctcttactgtcatgccatccgtaagatgcttttctgtgactggtgagtactcaaccaagtcattctgagaatagtgtatgcggcgaccgagttgctcttgcccggcgtcaatacgggataataccgcgccacatagcagaactttaaaagtgctcatcattggaaaacgttcttcggggcgaaaactctcaaggatcttaccgctgttgagatccagttcgatgtaacccactcgtgcacccaactgatcttcagcatcttttactttcaccagcgtttctgggtgagcaaaaacaggaaggcaaaatgccgcaaaaaagggaataagggcgacacggaaatgttgaatactcatactcttcctttttcaatattattgaagcatttatcagggttattgtctcatgagcggatacatatttgaatgtatttagaaaaataaacaaataggggttccgcgcacatttccccgaaaagtgccacctgacgcgccctgtagcggcgcattaagcgcggcgggtgtggtggttacgcgcagcgtgaccgctacacttgccagcgccctagcgcccgctcctttcgctttcttcccttcctttctcgccacgttcgccggctttccccgtcaagctctaaatcgggggctccctttagggttccgatttagtgctttacggcacctcgaccccaaaaaacttgattagggtgatggttcacgtagtgggccatcgccctgatagacggtttttcgccctttgacgttggagtccacgttctttaatagtggactcttgttccaaactggaacaacactcaaccctatctcggtctattcttttgatttataagggattttgccgatttcggcctattggttaaaaaatgagctgatttaacaaaaatttaacgcgaattttaacaaaatattaacgtttacaatttcccattcgccattcaggctgcgcaactgttgggaagggcgatcggtgcgggcctcttcgctattacgcca